European Patent Application EP 4 159 757 A1, published April 5, 2023. Title: SARS-COV-2 SPIKE PROTEIN BINDING MOLECULE AND APPLICATION THEREOF. Applicant: SHENZHEN IMMUNOTHERAPY BIOTECH CO., LTD. The sequence listing filed with the application follows.

SEQUENCE LISTING (143 sequences)

SEQ ID NO: 1 - protein, 8 aa, CDR1
GLSLEHYA

SEQ ID NO: 2 - protein, 8 aa, CDR2
ISDSGATR

SEQ ID NO: 3 - protein, 20 aa, CDR3
SATPGAFRTCAFRDFSHLAN

SEQ ID NO: 4 - protein, 8 aa, CDR1
GLSLEHYA

SEQ ID NO: 5 - protein, 8 aa, CDR2
IDSSGGST

SEQ ID NO: 6 - protein, 19 aa, CDR3
AALQGSYYYTSLHQTEYDY

SEQ ID NO: 7 - protein, 8 aa, CDR1
GFTLDSYA

SEQ ID NO: 8 - protein, 8 aa, CDR2
ITKHGGTT

SEQ ID NO: 9 - protein, 20 aa, CDR3
AADHRALRFGCAVVPGPYDY

SEQ ID NO: 10 - protein, 8 aa, CDR1
GLTLNNNT

SEQ ID NO: 11 - protein, 8 aa, CDR2
ISPSGIVT

SEQ ID NO: 12 - protein, 16 aa, CDR3
AVLQWNGAGLPSPLGS

SEQ ID NO: 13 - protein, 8 aa, CDR1
GFTLGNYE

SEQ ID NO: 14 - protein, 8 aa, CDR2
ISRSGVIF

SEQ ID NO: 15 - protein, 22 aa, CDR3
AARFRAGLVQSLCQSTPEFYQD

SEQ ID NO: 16 - protein, 8 aa, CDR1
GFTLGNYA

SEQ ID NO: 17 - protein, 8 aa, CDR2
ISLSGDII

SEQ ID NO: 18 - protein, 22 aa, CDR3
AAPFPSLLYCSLCPSNPEFCRH

SEQ ID NO: 19 - protein, 8 aa, CDR1
GFSLDGYA

SEQ ID NO: 20 - protein, 8 aa, CDR2
IGRLGTTT

SEQ ID NO: 21 - protein, 18 aa, CDR3
AAKRSTWFGCSTLDDYDY

SEQ ID NO: 22 - protein, 8 aa, CDR1
GFTLDRYA

SEQ ID NO: 23 - protein, 7 aa, CDR2
ISSGGTT

SEQ ID NO: 24 - protein, 19 aa, CDR3
AAGTQLRYGCSRQARRYDY

SEQ ID NO: 25 - protein, 8 aa, CDR1
GFTLDYYA

SEQ ID NO: 26 - protein, 8 aa, CDR2
ISSSGTST

SEQ ID NO: 27 - protein, 19 aa, CDR3
AALQGSYYYTSLHQTEYDY

SEQ ID NO: 28 - protein, 8 aa, CDR1
GATSDIYA

SEQ ID NO: 29 - protein, 8 aa, CDR2
ISPSGGST

SEQ ID NO: 30 - protein, 19 aa, CDR3
AAASPSWHYCSGYEHEYDD

SEQ ID NO: 31 - protein, 8 aa, CDR1
GFTLDYYA

SEQ ID NO: 32 - protein, 8 aa, CDR2
ISPSGTST

SEQ ID NO: 33 - protein, 19 aa, CDR3
AAANPSYYYCSGYPHEYDD

SEQ ID NO: 34 - protein, 8 aa, CDR1
GFTFHYYA

SEQ ID NO: 35 - protein, 8 aa, CDR2
ISSGGGRT

SEQ ID NO: 36 - protein, 19 aa, CDR3
AALQGSLHYCSGLVGEYEY

SEQ ID NO: 37 - protein, 8 aa, CDR1
FKSYHIAW

SEQ ID NO: 38 - protein, 8 aa, CDR2
SLTGASIT

SEQ ID NO: 39 - protein, 20 aa, CDR3
AARDYASSLYCSRNEAMYAY

SEQ ID NO: 40 - protein, 8 aa, CDR1
GFRLGGYA

SEQ ID NO: 41 - protein, 8 aa, CDR2
ISGSGIIS

SEQ ID NO: 42 - protein, 24 aa, CDR3
AAPSGSSYGSRRLPCGIDSQDYQT

SEQ ID NO: 43 - protein, 8 aa, CDR1
FDDFAIGW

SEQ ID NO: 44 - protein, 8 aa, CDR2
SARGIVNT

SEQ ID NO: 45 - protein, 20 aa, CDR3
AALVGLNDRSLPHEAEEYDY

SEQ ID NO: 46 - protein, 8 aa, CDR1
GFTFDDYS

SEQ ID NO: 47 - protein, 8 aa, CDR2
FSSLDGST

SEQ ID NO: 48 - protein, 18 aa, CDR3
AATRGSSWYWYRPSEYDY

SEQ ID NO: 49 - protein, 8 aa, CDR1
GHTGSTYI

SEQ ID NO: 50 - protein, 8 aa, CDR2
ISRSGILR

SEQ ID NO: 51 - protein, 19 aa, CDR3
AARDSLTGVIGNTPGEYDY

SEQ ID NO: 52 - protein, 8 aa, CDR1
GRTVSSYV

SEQ ID NO: 53 - protein, 8 aa, CDR2
ISRSGIIT

SEQ ID NO: 54 - protein, 17 aa, CDR3
AAAQTQVLPTEDRSYDY

SEQ ID NO: 55 - protein, 8 aa, CDR1
GRTFTRYP

SEQ ID NO: 56 - protein, 8 aa, CDR2
ISGSGIIT

SEQ ID NO: 57 - protein, 19 aa, CDR3
AVDNAPTSSLPLTPGEYDY

SEQ ID NO: 58 - protein, 8 aa, CDR1
GRTFSSYA

SEQ ID NO: 59 - protein, 7 aa, CDR2
ISSGGIT

SEQ ID NO: 60 - protein, 18 aa, CDR3
AANRGRFTGWRSLTDYTY

SEQ ID NO: 61 - protein, 8 aa, CDR1
GRTFSTYA

SEQ ID NO: 62 - protein, 8 aa, CDR2
ISPSRIIT

SEQ ID NO: 63 - protein, 19 aa, CDR3
AADSSYGGRLGRRIDDYEY

SEQ ID NO: 64 - protein, 8 aa, CDR1
GSGVSTGS

SEQ ID NO: 65 - protein, 7 aa, CDR2
YTSVGSI

SEQ ID NO: 66 - protein, 10 aa, CDR3
AFFVPFGDTY

SEQ ID NO: 67 - protein, 8 aa, CDR1
ASGRTSST

SEQ ID NO: 68 - protein, 8 aa, CDR2
ITWSGGST

SEQ ID NO: 69 - protein, 17 aa, CDR3
AAGLSPLMLTASRRYEY

SEQ ID NO: 70 - protein, 8 aa, CDR1
GRTVSMYA

SEQ ID NO: 71 - protein, 8 aa, CDR2
ISRSGRST

SEQ ID NO: 72 - protein, 20 aa, CDR3
AARDGGLHYALYVEASHYNY

SEQ ID NO: 73 - protein, 8 aa, CDR1
GFTFSSYA

SEQ ID NO: 74 - protein, 8 aa, CDR2
LDVTGRST

SEQ ID NO: 75 - protein, 20 aa, CDR3
AAVYTPFRFAFKTDPDRQDH

SEQ ID NO: 76 - protein, 8 aa, CDR1
GRTFGTYR

SEQ ID NO: 77 - protein, 8 aa, CDR2
IFWSGGGA

SEQ ID NO: 78 - protein, 12 aa, CDR3
AARAPTTQEYDY

SEQ ID NO: 79 - protein, 8 aa, CDR1
GRTLSTYE

SEQ ID NO: 80 - protein, 8 aa, CDR2
VTPTGFGT

SEQ ID NO: 81 - protein, 16 aa, CDR3
AGSGKGLGSLQRSPDD

SEQ ID NO: 82 - protein, 127 aa, VHH1
QLQLVESGGDLVQPGESLRLSCVASGLSLEHYAIGWFRQAPGKEREGVSCISDSGATRSYADSVRGRFTISRENAKNAVYLEMNSLKPEDTAVYYCSATPGAFRTCAFRDFSHLANWGQGTQVTVSS

SEQ ID NO: 83 - protein, 126 aa, VHH2
QLQLVESGGDLVQPGESLRLSCVASGLSLEHYAIGWFRQAPGKEREGVSCIDSSGGSTSYADSVRGRFTISRENAKNAVYLEMNSLKPEDTAVYYCAALQGSYYYTSLHQTEYDYWGQGTQVTVSS

SEQ ID NO: 84 - protein, 127 aa, VHH3
QLQLVESGGDLVQPGESLRLSCVASGFTLDSYAIGWFRQAPGKEREGVSCITKHGGTTSYADSVRGRFTISRENAKNAVYLEMNSLKPEDTAVYYCAADHRALRFGCAVVPGPYDYWGQGTQVTVSS

SEQ ID NO: 85 - protein, 123 aa, VHH4
QLQLVESGGDLVQPGESLRLSCVASGLTLNNNTIGWFRQAPGKEREGVSCISPSGIVTSYADSVRGRFTISRENAKNAVYLEMNSLKPEDTAVYYCAVLQWNGAGLPSPLGSWGQGTQVTVSS

SEQ ID NO: 86 - protein, 129 aa, VHH5
QLQLVESGGDLVQPGESLRLSCVASGFTLGNYEIGWFRQAPGKEREGVSCISRSGVIFSYADSVRGRFTISRENAKNAVYLEMNSLKPEDTAVYYCAARFRAGLVQSLCQSTPEFYQDWGQGTQVTVSS

SEQ ID NO: 87 - protein, 129 aa, VHH6
QLQLVESGGDLVQPGESLRLSCVASGFTLGNYAIGWFRQAPGKEREGVSCISLSGDIISYADSVRGRFTISRENAKNAVYLEMNSLKPEDTAVYYCAAPFPSLLYCSLCPSNPEFCRHWGQGTQVTVSS

SEQ ID NO: 88 - protein, 125 aa, VHH7
QLQLVESGGDLVQPGESLRLSCVASGFSLDGYAIGWFRQAPGKEREGVSCIGRLGTTTSYADSVRGRFTISRENAKNAVYLEMNSLKPEDTAVYYCAAKRSTWFGCSTLDDYDYWGQGTQVTVSS

SEQ ID NO: 89 - protein, 125 aa, VHH8
QLQLVESGGDLVQPGESLRLSCVASGFTLDRYAIGWFRQAPGKEREGVSCISSGGTTSYADSVRGRFTISRENAKNAVYLEMNSLKPEDTAVYYCAAGTQLRYGCSRQARRYDYWGQGTQVTVSS

SEQ ID NO: 90 - protein, 126 aa, VHH9
QLQLVESGGDLVQPGESLRLSCVASGFTLDYYAIGWFRQAPGKEREGVSCISSSGTSTSYADSVRGRFTISRENAKNAVYLEMNSLKPEDTAVYYCAALQGSYYYTSLHQTEYDYWGQGTQVTVSS

SEQ ID NO: 91 - protein, 126 aa, VHH10
QLQLVESGGDLVQPGESLRLSCVASGATSDIYAIGWFRQAPGKEREGVSCISPSGGSTSYADSVRGRFTISRENAKNAVYLEMNSLKPEDTAVYYCAAASPSWHYCSGYEHEYDDWGQGTQVTVSS

SEQ ID NO: 92 - protein, 126 aa, VHH11
QLQLVESGGDLVQPGESLRLSCVASGFTLDYYAIGWFRQAPGKEREGVSCISPSGTSTSYADSVRGRFTISRENAKNAVYLEMNSLKPEDTAVYYCAAANPSYYYCSGYPHEYDDWGQGTQVTVSS

SEQ ID NO: 93 - protein, 126 aa, VHH12
QLQLVESGGDLVQPGESLRLSCVASGFTFHYYAIGWFRQAPGKEREGVSCISSGGGRTSYADSVRGRFTISRENAKNAVYLEMNSLKPEDTAVYYCAALQGSLHYCSGLVGEYEYWGQGTQVTVSS

SEQ ID NO: 94 - protein, 127 aa, VHH13
QLQLVESGGDLVQPGESLRLSCVASFKSYHIAWIGWFRQAPGKEREGVSCSLTGASITSYADSVRGRFTISRENAKNAVYLEMNSLKPEDTAVYYCAARDYASSLYCSRNEAMYAYWGQGTQVTVSS

SEQ ID NO: 95 - protein, 131 aa, VHH14
QLQLVESGGDLVQPGESLRLSCVASGFRLGGYAIGWFRQAPGKEREGVSCISGSGIISSYADSVRGRFTISRENAKNAVYLEMNSLKPEDTAVYYCAAPSGSSYGSRRLPCGIDSQDYQTWGQGTQVTVSS

SEQ ID NO: 96 - protein, 127 aa, VHH15
QLQLVESGGDLVQPGESLRLSCVASFDDFAIGWIGWFRQAPGKEREGVSCSARGIVNTSYADSVRGRFTISRENAKNAVYLEMNSLKPEDTAVYYCAALVGLNDRSLPHEAEEYDYWGQGTQVTVSS

SEQ ID NO: 97 - protein, 125 aa, VHH16
QLQLVESGGDLVQPGESLRLSCVASGFTFDDYSIGWFRQAPGKEREGVSCFSSLDGSTSYADSVRGRFTISRENAKNAVYLEMNSLKPEDTAVYYCAATRGSSWYWYRPSEYDYWGQGTQVTVSS

SEQ ID NO: 98 - protein, 126 aa, VHH17
QLQLVESGGDLVQPGESLRLSCVASGHTGSTYIIGWFRQAPGKEREGVSCISRSGILRSYADSVRGRFTISRENAKNAVYLEMNSLKPEDTAVYYCAARDSLTGVIGNTPGEYDYWGQGTQVTVSS

SEQ ID NO: 99 - protein, 124 aa, VHH18
QLQLVESGGDLVQPGESLRLSCVASGRTVSSYVIGWFRQAPGKEREGVSCISRSGIITSYADSVRGRFTISRENAKNAVYLEMNSLKPEDTAVYYCAAAQTQVLPTEDRSYDYWGQGTQVTVSS

SEQ ID NO: 100 - protein, 126 aa, VHH19
QLQLVESGGDLVQPGESLRLSCVASGRTFTRYPIGWFRQAPGKEREGVSCISGSGIITSYADSVRGRFTISRENAKNAVYLEMNSLKPEDTAVYYCAVDNAPTSSLPLTPGEYDYWGQGTQVTVSS

SEQ ID NO: 101 - protein, 124 aa, VHH20
QLQLVESGGDLVQPGESLRLSCVASGRTFSSYAIGWFRQAPGKEREGVSCISSGGITSYADSVRGRFTISRENAKNAVYLEMNSLKPEDTAVYYCAANRGRFTGWRSLTDYTYWGQGTQVTVSS

SEQ ID NO: 102 - protein, 126 aa, VHH21
QLQLVESGGDLVQPGESLRLSCVASGRTFSTYAIGWFRQAPGKEREGVSCISPSRIITSYADSVRGRFTISRENAKNAVYLEMNSLKPEDTAVYYCAADSSYGGRLGRRIDDYEYWGQGTQVTVSS

SEQ ID NO: 103 - protein, 116 aa, VHH22
QLQLVESGGDLVQPGESLRLSCVASGSGVSTGSIGWFRQAPGKEREGVSCYTSVGSISYADSVRGRFTISRENAKNAVYLEMNSLKPEDTAVYYCAFFVPFGDTYWGQGTQVTVSS

SEQ ID NO: 104 - protein, 124 aa, VHH23
QLQLVESGGDLVQPGESLRLSCVASASGRTSSTIGWFRQAPGKEREGVSCITWSGGSTSYADSVRGRFTISRENAKNAVYLEMNSLKPEDTAVYYCAAGLSPLMLTASRRYEYWGQGTQVTVSS

SEQ ID NO: 105 - protein, 127 aa, VHH24
QLQLVESGGDLVQPGESLRLSCVASGRTVSMYAIGWFRQAPGKEREGVSCISRSGRSTSYADSVRGRFTISRENAKNAVYLEMNSLKPEDTAVYYCAARDGGLHYALYVEASHYNYWGQGTQVTVSS

SEQ ID NO: 106 - protein, 127 aa, VHH25
QLQLVESGGDLVQPGESLRLSCVASGFTFSSYAIGWFRQAPGKEREGVSCLDVTGRSTSYADSVRGRFTISRENAKNAVYLEMNSLKPEDTAVYYCAAVYTPFRFAFKTDPDRQDHWGQGTQVTVSS

SEQ ID NO: 107 - protein, 119 aa, VHH26
QLQLVESGGDLVQPGESLRLSCVASGRTFGTYRIGWFRQAPGKEREGVSCIFWSGGGASYADSVRGRFTISRENAKNAVYLEMNSLKPEDTAVYYCAARAPTTQEYDYWGQGTQVTVSS

SEQ ID NO: 108 - protein, 123 aa, VHH27
QLQLVESGGDLVQPGESLRLSCVASGRTLSTYEIGWFRQAPGKEREGVSCVTPTGFGTSYADSVRGRFTISRENAKNAVYLEMNSLKPEDTAVYYCAGSGKGLGSLQRSPDDWGQGTQVTVSS

SEQ ID NO: 109 - protein, 232 aa, Fc
EPKSSDKTHTCPPCPAPELLGGPSVFLFPPKPKDTLMISRTPEVTCVVVDVSHEDPEVKFNWYVDGVEVHNAKTKPREEQYNSTYRVVSVLTVLHQDWLNGKEYKCKVSNKALPAPIEKTISKAKGQPREPQVYTLPPSRDELTKNQVSLTCLVKGFYPSDIAVEWESNGQPENNYKTTPPVLDSDGSFFLYSKLTVDKSRWQQGNVFSCSVMHEALHNHYTQKSLSLSPGK

SEQ ID NO: 110 - protein, 359 aa, VHH1-Fc
QLQLVESGGDLVQPGESLRLSCVASGLSLEHYAIGWFRQAPGKEREGVSCISDSGATRSYADSVRGRFTISRENAKNAVYLEMNSLKPEDTAVYYCSATPGAFRTCAFRDFSHLANWGQGTQVTVSSEPKSSDKTHTCPPCPAPELLGGPSVFLFPPKPKDTLMISRTPEVTCVVVDVSHEDPEVKFNWYVDGVEVHNAKTKPREEQYNSTYRVVSVLTVLHQDWLNGKEYKCKVSNKALPAPIEKTISKAKGQPREPQVYTLPPSRDELTKNQVSLTCLVKGFYPSDIAVEWESNGQPENNYKTTPPVLDSDGSFFLYSKLTVDKSRWQQGNVFSCSVMHEALHNHYTQKSLSLSPGK

SEQ ID NO: 111 - protein, 358 aa, VHH2-Fc
QLQLVESGGDLVQPGESLRLSCVASGLSLEHYAIGWFRQAPGKEREGVSCIDSSGGSTSYADSVRGRFTISRENAKNAVYLEMNSLKPEDTAVYYCAALQGSYYYTSLHQTEYDYWGQGTQVTVSSEPKSSDKTHTCPPCPAPELLGGPSVFLFPPKPKDTLMISRTPEVTCVVVDVSHEDPEVKFNWYVDGVEVHNAKTKPREEQYNSTYRVVSVLTVLHQDWLNGKEYKCKVSNKALPAPIEKTISKAKGQPREPQVYTLPPSRDELTKNQVSLTCLVKGFYPSDIAVEWESNGQPENNYKTTPPVLDSDGSFFLYSKLTVDKSRWQQGNVFSCSVMHEALHNHYTQKSLSLSPGK

SEQ ID NO: 112 - protein, 359 aa, VHH3-Fc
QLQLVESGGDLVQPGESLRLSCVASGFTLDSYAIGWFRQAPGKEREGVSCITKHGGTTSYADSVRGRFTISRENAKNAVYLEMNSLKPEDTAVYYCAADHRALRFGCAVVPGPYDYWGQGTQVTVSSEPKSSDKTHTCPPCPAPELLGGPSVFLFPPKPKDTLMISRTPEVTCVVVDVSHEDPEVKFNWYVDGVEVHNAKTKPREEQYNSTYRVVSVLTVLHQDWLNGKEYKCKVSNKALPAPIEKTISKAKGQPREPQVYTLPPSRDELTKNQVSLTCLVKGFYPSDIAVEWESNGQPENNYKTTPPVLDSDGSFFLYSKLTVDKSRWQQGNVFSCSVMHEALHNHYTQKSLSLSPGK

SEQ ID NO: 113 - protein, 355 aa, VHH4-Fc
QLQLVESGGDLVQPGESLRLSCVASGLTLNNNTIGWFRQAPGKEREGVSCISPSGIVTSYADSVRGRFTISRENAKNAVYLEMNSLKPEDTAVYYCAVLQWNGAGLPSPLGSWGQGTQVTVSSEPKSSDKTHTCPPCPAPELLGGPSVFLFPPKPKDTLMISRTPEVTCVVVDVSHEDPEVKFNWYVDGVEVHNAKTKPREEQYNSTYRVVSVLTVLHQDWLNGKEYKCKVSNKALPAPIEKTISKAKGQPREPQVYTLPPSRDELTKNQVSLTCLVKGFYPSDIAVEWESNGQPENNYKTTPPVLDSDGSFFLYSKLTVDKSRWQQGNVFSCSVMHEALHNHYTQKSLSLSPGK

SEQ ID NO: 114 - protein, 361 aa, VHH5-Fc
QLQLVESGGDLVQPGESLRLSCVASGFTLGNYEIGWFRQAPGKEREGVSCISRSGVIFSYADSVRGRFTISRENAKNAVYLEMNSLKPEDTAVYYCAARFRAGLVQSLCQSTPEFYQDWGQGTQVTVSSEPKSSDKTHTCPPCPAPELLGGPSVFLFPPKPKDTLMISRTPEVTCVVVDVSHEDPEVKFNWYVDGVEVHNAKTKPREEQYNSTYRVVSVLTVLHQDWLNGKEYKCKVSNKALPAPIEKTISKAKGQPREPQVYTLPPSRDELTKNQVSLTCLVKGFYPSDIAVEWESNGQPENNYKTTPPVLDSDGSFFLYSKLTVDKSRWQQGNVFSCSVMHEALHNHYTQKSLSLSPGK

SEQ ID NO: 115 - protein, 361 aa, VHH6-Fc
QLQLVESGGDLVQPGESLRLSCVASGFTLGNYAIGWFRQAPGKEREGVSCISLSGDIISYADSVRGRFTISRENAKNAVYLEMNSLKPEDTAVYYCAAPFPSLLYCSLCPSNPEFCRHWGQGTQVTVSSEPKSSDKTHTCPPCPAPELLGGPSVFLFPPKPKDTLMISRTPEVTCVVVDVSHEDPEVKFNWYVDGVEVHNAKTKPREEQYNSTYRVVSVLTVLHQDWLNGKEYKCKVSNKALPAPIEKTISKAKGQPREPQVYTLPPSRDELTKNQVSLTCLVKGFYPSDIAVEWESNGQPENNYKTTPPVLDSDGSFFLYSKLTVDKSRWQQGNVFSCSVMHEALHNHYTQKSLSLSPGK

SEQ ID NO: 116 - protein, 357 aa, VHH7-Fc
QLQLVESGGDLVQPGESLRLSCVASGFSLDGYAIGWFRQAPGKEREGVSCIGRLGTTTSYADSVRGRFTISRENAKNAVYLEMNSLKPEDTAVYYCAAKRSTWFGCSTLDDYDYWGQGTQVTVSSEPKSSDKTHTCPPCPAPELLGGPSVFLFPPKPKDTLMISRTPEVTCVVVDVSHEDPEVKFNWYVDGVEVHNAKTKPREEQYNSTYRVVSVLTVLHQDWLNGKEYKCKVSNKALPAPIEKTISKAKGQPREPQVYTLPPSRDELTKNQVSLTCLVKGFYPSDIAVEWESNGQPENNYKTTPPVLDSDGSFFLYSKLTVDKSRWQQGNVFSCSVMHEALHNHYTQKSLSLSPGK

SEQ ID NO: 117 - protein, 357 aa, VHH8-Fc
QLQLVESGGDLVQPGESLRLSCVASGFTLDRYAIGWFRQAPGKEREGVSCISSGGTTSYADSVRGRFTISRENAKNAVYLEMNSLKPEDTAVYYCAAGTQLRYGCSRQARRYDYWGQGTQVTVSSEPKSSDKTHTCPPCPAPELLGGPSVFLFPPKPKDTLMISRTPEVTCVVVDVSHEDPEVKFNWYVDGVEVHNAKTKPREEQYNSTYRVVSVLTVLHQDWLNGKEYKCKVSNKALPAPIEKTISKAKGQPREPQVYTLPPSRDELTKNQVSLTCLVKGFYPSDIAVEWESNGQPENNYKTTPPVLDSDGSFFLYSKLTVDKSRWQQGNVFSCSVMHEALHNHYTQKSLSLSPGK

SEQ ID NO: 118 - protein, 358 aa, VHH9-Fc
QLQLVESGGDLVQPGESLRLSCVASGFTLDYYAIGWFRQAPGKEREGVSCISSSGTSTSYADSVRGRFTISRENAKNAVYLEMNSLKPEDTAVYYCAALQGSYYYTSLHQTEYDYWGQGTQVTVSSEPKSSDKTHTCPPCPAPELLGGPSVFLFPPKPKDTLMISRTPEVTCVVVDVSHEDPEVKFNWYVDGVEVHNAKTKPREEQYNSTYRVVSVLTVLHQDWLNGKEYKCKVSNKALPAPIEKTISKAKGQPREPQVYTLPPSRDELTKNQVSLTCLVKGFYPSDIAVEWESNGQPENNYKTTPPVLDSDGSFFLYSKLTVDKSRWQQGNVFSCSVMHEALHNHYTQKSLSLSPGK

SEQ ID NO: 119 - protein, 358 aa, VHH10-Fc
QLQLVESGGDLVQPGESLRLSCVASGATSDIYAIGWFRQAPGKEREGVSCISPSGGSTSYADSVRGRFTISRENAKNAVYLEMNSLKPEDTAVYYCAAASPSWHYCSGYEHEYDDWGQGTQVTVSSEPKSSDKTHTCPPCPAPELLGGPSVFLFPPKPKDTLMISRTPEVTCVVVDVSHEDPEVKFNWYVDGVEVHNAKTKPREEQYNSTYRVVSVLTVLHQDWLNGKEYKCKVSNKALPAPIEKTISKAKGQPREPQVYTLPPSRDELTKNQVSLTCLVKGFYPSDIAVEWESNGQPENNYKTTPPVLDSDGSFFLYSKLTVDKSRWQQGNVFSCSVMHEALHNHYTQKSLSLSPGK

SEQ ID NO: 120 - protein, 358 aa, VHH11-Fc
QLQLVESGGDLVQPGESLRLSCVASGFTLDYYAIGWFRQAPGKEREGVSCISPSGTSTSYADSVRGRFTISRENAKNAVYLEMNSLKPEDTAVYYCAAANPSYYYCSGYPHEYDDWGQGTQVTVSSEPKSSDKTHTCPPCPAPELLGGPSVFLFPPKPKDTLMISRTPEVTCVVVDVSHEDPEVKFNWYVDGVEVHNAKTKPREEQYNSTYRVVSVLTVLHQDWLNGKEYKCKVSNKALPAPIEKTISKAKGQPREPQVYTLPPSRDELTKNQVSLTCLVKGFYPSDIAVEWESNGQPENNYKTTPPVLDSDGSFFLYSKLTVDKSRWQQGNVFSCSVMHEALHNHYTQKSLSLSPGK

SEQ ID NO: 121 - protein, 358 aa, VHH12-Fc
QLQLVESGGDLVQPGESLRLSCVASGFTFHYYAIGWFRQAPGKEREGVSCISSGGGRTSYADSVRGRFTISRENAKNAVYLEMNSLKPEDTAVYYCAALQGSLHYCSGLVGEYEYWGQGTQVTVSSEPKSSDKTHTCPPCPAPELLGGPSVFLFPPKPKDTLMISRTPEVTCVVVDVSHEDPEVKFNWYVDGVEVHNAKTKPREEQYNSTYRVVSVLTVLHQDWLNGKEYKCKVSNKALPAPIEKTISKAKGQPREPQVYTLPPSRDELTKNQVSLTCLVKGFYPSDIAVEWESNGQPENNYKTTPPVLDSDGSFFLYSKLTVDKSRWQQGNVFSCSVMHEALHNHYTQKSLSLSPGK

SEQ ID NO: 122 - protein, 359 aa, VHH13-Fc
QLQLVESGGDLVQPGESLRLSCVASFKSYHIAWIGWFRQAPGKEREGVSCSLTGASITSYADSVRGRFTISRENAKNAVYLEMNSLKPEDTAVYYCAARDYASSLYCSRNEAMYAYWGQGTQVTVSSEPKSSDKTHTCPPCPAPELLGGPSVFLFPPKPKDTLMISRTPEVTCVVVDVSHEDPEVKFNWYVDGVEVHNAKTKPREEQYNSTYRVVSVLTVLHQDWLNGKEYKCKVSNKALPAPIEKTISKAKGQPREPQVYTLPPSRDELTKNQVSLTCLVKGFYPSDIAVEWESNGQPENNYKTTPPVLDSDGSFFLYSKLTVDKSRWQQGNVFSCSVMHEALHNHYTQKSLSLSPGK

SEQ ID NO: 123 - protein, 363 aa, VHH14-Fc
QLQLVESGGDLVQPGESLRLSCVASGFRLGGYAIGWFRQAPGKEREGVSCISGSGIISSYADSVRGRFTISRENAKNAVYLEMNSLKPEDTAVYYCAAPSGSSYGSRRLPCGIDSQDYQTWGQGTQVTVSSEPKSSDKTHTCPPCPAPELLGGPSVFLFPPKPKDTLMISRTPEVTCVVVDVSHEDPEVKFNWYVDGVEVHNAKTKPREEQYNSTYRVVSVLTVLHQDWLNGKEYKCKVSNKALPAPIEKTISKAKGQPREPQVYTLPPSRDELTKNQVSLTCLVKGFYPSDIAVEWESNGQPENNYKTTPPVLDSDGSFFLYSKLTVDKSRWQQGNVFSCSVMHEALHNHYTQKSLSLSPGK

SEQ ID NO: 124 - protein, 359 aa, VHH15-Fc
QLQLVESGGDLVQPGESLRLSCVASFDDFAIGWIGWFRQAPGKEREGVSCSARGIVNTSYADSVRGRFTISRENAKNAVYLEMNSLKPEDTAVYYCAALVGLNDRSLPHEAEEYDYWGQGTQVTVSSEPKSSDKTHTCPPCPAPELLGGPSVFLFPPKPKDTLMISRTPEVTCVVVDVSHEDPEVKFNWYVDGVEVHNAKTKPREEQYNSTYRVVSVLTVLHQDWLNGKEYKCKVSNKALPAPIEKTISKAKGQPREPQVYTLPPSRDELTKNQVSLTCLVKGFYPSDIAVEWESNGQPENNYKTTPPVLDSDGSFFLYSKLTVDKSRWQQGNVFSCSVMHEALHNHYTQKSLSLSPGK

SEQ ID NO: 125 - protein, 357 aa, VHH16-Fc
QLQLVESGGDLVQPGESLRLSCVASGFTFDDYSIGWFRQAPGKEREGVSCFSSLDGSTSYADSVRGRFTISRENAKNAVYLEMNSLKPEDTAVYYCAATRGSSWYWYRPSEYDYWGQGTQVTVSSEPKSSDKTHTCPPCPAPELLGGPSVFLFPPKPKDTLMISRTPEVTCVVVDVSHEDPEVKFNWYVDGVEVHNAKTKPREEQYNSTYRVVSVLTVLHQDWLNGKEYKCKVSNKALPAPIEKTISKAKGQPREPQVYTLPPSRDELTKNQVSLTCLVKGFYPSDIAVEWESNGQPENNYKTTPPVLDSDGSFFLYSKLTVDKSRWQQGNVFSCSVMHEALHNHYTQKSLSLSPGK

SEQ ID NO: 126 - protein, 358 aa, VHH17-Fc
QLQLVESGGDLVQPGESLRLSCVASGHTGSTYIIGWFRQAPGKEREGVSCISRSGILRSYADSVRGRFTISRENAKNAVYLEMNSLKPEDTAVYYCAARDSLTGVIGNTPGEYDYWGQGTQVTVSSEPKSSDKTHTCPPCPAPELLGGPSVFLFPPKPKDTLMISRTPEVTCVVVDVSHEDPEVKFNWYVDGVEVHNAKTKPREEQYNSTYRVVSVLTVLHQDWLNGKEYKCKVSNKALPAPIEKTISKAKGQPREPQVYTLPPSRDELTKNQVSLTCLVKGFYPSDIAVEWESNGQPENNYKTTPPVLDSDGSFFLYSKLTVDKSRWQQGNVFSCSVMHEALHNHYTQKSLSLSPGK

SEQ ID NO: 127 - protein, 356 aa, VHH18-Fc
QLQLVESGGDLVQPGESLRLSCVASGRTVSSYVIGWFRQAPGKEREGVSCISRSGIITSYADSVRGRFTISRENAKNAVYLEMNSLKPEDTAVYYCAAAQTQVLPTEDRSYDYWGQGTQVTVSSEPKSSDKTHTCPPCPAPELLGGPSVFLFPPKPKDTLMISRTPEVTCVVVDVSHEDPEVKFNWYVDGVEVHNAKTKPREEQYNSTYRVVSVLTVLHQDWLNGKEYKCKVSNKALPAPIEKTISKAKGQPREPQVYTLPPSRDELTKNQVSLTCLVKGFYPSDIAVEWESNGQPENNYKTTPPVLDSDGSFFLYSKLTVDKSRWQQGNVFSCSVMHEALHNHYTQKSLSLSPGK

SEQ ID NO: 128 - protein, 358 aa, VHH19-Fc
QLQLVESGGDLVQPGESLRLSCVASGRTFTRYPIGWFRQAPGKEREGVSCISGSGIITSYADSVRGRFTISRENAKNAVYLEMNSLKPEDTAVYYCAVDNAPTSSLPLTPGEYDYWGQGTQVTVSSEPKSSDKTHTCPPCPAPELLGGPSVFLFPPKPKDTLMISRTPEVTCVVVDVSHEDPEVKFNWYVDGVEVHNAKTKPREEQYNSTYRVVSVLTVLHQDWLNGKEYKCKVSNKALPAPIEKTISKAKGQPREPQVYTLPPSRDELTKNQVSLTCLVKGFYPSDIAVEWESNGQPENNYKTTPPVLDSDGSFFLYSKLTVDKSRWQQGNVFSCSVMHEALHNHYTQKSLSLSPGK

SEQ ID NO: 129 - protein, 356 aa, VHH20-Fc
QLQLVESGGDLVQPGESLRLSCVASGRTFSSYAIGWFRQAPGKEREGVSCISSGGITSYADSVRGRFTISRENAKNAVYLEMNSLKPEDTAVYYCAANRGRFTGWRSLTDYTYWGQGTQVTVSSEPKSSDKTHTCPPCPAPELLGGPSVFLFPPKPKDTLMISRTPEVTCVVVDVSHEDPEVKFNWYVDGVEVHNAKTKPREEQYNSTYRVVSVLTVLHQDWLNGKEYKCKVSNKALPAPIEKTISKAKGQPREPQVYTLPPSRDELTKNQVSLTCLVKGFYPSDIAVEWESNGQPENNYKTTPPVLDSDGSFFLYSKLTVDKSRWQQGNVFSCSVMHEALHNHYTQKSLSLSPGK

SEQ ID NO: 130 - protein, 358 aa, VHH21-Fc
QLQLVESGGDLVQPGESLRLSCVASGRTFSTYAIGWFRQAPGKEREGVSCISPSRIITSYADSVRGRFTISRENAKNAVYLEMNSLKPEDTAVYYCAADSSYGGRLGRRIDDYEYWGQGTQVTVSSEPKSSDKTHTCPPCPAPELLGGPSVFLFPPKPKDTLMISRTPEVTCVVVDVSHEDPEVKFNWYVDGVEVHNAKTKPREEQYNSTYRVVSVLTVLHQDWLNGKEYKCKVSNKALPAPIEKTISKAKGQPREPQVYTLPPSRDELTKNQVSLTCLVKGFYPSDIAVEWESNGQPENNYKTTPPVLDSDGSFFLYSKLTVDKSRWQQGNVFSCSVMHEALHNHYTQKSLSLSPGK

SEQ ID NO: 131 - protein, 348 aa, VHH22-Fc
QLQLVESGGDLVQPGESLRLSCVASGSGVSTGSIGWFRQAPGKEREGVSCYTSVGSISYADSVRGRFTISRENAKNAVYLEMNSLKPEDTAVYYCAFFVPFGDTYWGQGTQVTVSSEPKSSDKTHTCPPCPAPELLGGPSVFLFPPKPKDTLMISRTPEVTCVVVDVSHEDPEVKFNWYVDGVEVHNAKTKPREEQYNSTYRVVSVLTVLHQDWLNGKEYKCKVSNKALPAPIEKTISKAKGQPREPQVYTLPPSRDELTKNQVSLTCLVKGFYPSDIAVEWESNGQPENNYKTTPPVLDSDGSFFLYSKLTVDKSRWQQGNVFSCSVMHEALHNHYTQKSLSLSPGK

SEQ ID NO: 132 - protein, 356 aa, VHH23-Fc
QLQLVESGGDLVQPGESLRLSCVASASGRTSSTIGWFRQAPGKEREGVSCITWSGGSTSYADSVRGRFTISRENAKNAVYLEMNSLKPEDTAVYYCAAGLSPLMLTASRRYEYWGQGTQVTVSSEPKSSDKTHTCPPCPAPELLGGPSVFLFPPKPKDTLMISRTPEVTCVVVDVSHEDPEVKFNWYVDGVEVHNAKTKPREEQYNSTYRVVSVLTVLHQDWLNGKEYKCKVSNKALPAPIEKTISKAKGQPREPQVYTLPPSRDELTKNQVSLTCLVKGFYPSDIAVEWESNGQPENNYKTTPPVLDSDGSFFLYSKLTVDKSRWQQGNVFSCSVMHEALHNHYTQKSLSLSPGK

SEQ ID NO: 133 - protein, 359 aa, VHH24-Fc
QLQLVESGGDLVQPGESLRLSCVASGRTVSMYAIGWFRQAPGKEREGVSCISRSGRSTSYADSVRGRFTISRENAKNAVYLEMNSLKPEDTAVYYCAARDGGLHYALYVEASHYNYWGQGTQVTVSSEPKSSDKTHTCPPCPAPELLGGPSVFLFPPKPKDTLMISRTPEVTCVVVDVSHEDPEVKFNWYVDGVEVHNAKTKPREEQYNSTYRVVSVLTVLHQDWLNGKEYKCKVSNKALPAPIEKTISKAKGQPREPQVYTLPPSRDELTKNQVSLTCLVKGFYPSDIAVEWESNGQPENNYKTTPPVLDSDGSFFLYSKLTVDKSRWQQGNVFSCSVMHEALHNHYTQKSLSLSPGK

SEQ ID NO: 134 - protein, 359 aa, VHH25-Fc
QLQLVESGGDLVQPGESLRLSCVASGFTFSSYAIGWFRQAPGKEREGVSCLDVTGRSTSYADSVRGRFTISRENAKNAVYLEMNSLKPEDTAVYYCAAVYTPFRFAFKTDPDRQDHWGQGTQVTVSSEPKSSDKTHTCPPCPAPELLGGPSVFLFPPKPKDTLMISRTPEVTCVVVDVSHEDPEVKFNWYVDGVEVHNAKTKPREEQYNSTYRVVSVLTVLHQDWLNGKEYKCKVSNKALPAPIEKTISKAKGQPREPQVYTLPPSRDELTKNQVSLTCLVKGFYPSDIAVEWESNGQPENNYKTTPPVLDSDGSFFLYSKLTVDKSRWQQGNVFSCSVMHEALHNHYTQKSLSLSPGK

SEQ ID NO: 135 - protein, 351 aa, VHH26-Fc
QLQLVESGGDLVQPGESLRLSCVASGRTFGTYRIGWFRQAPGKEREGVSCIFWSGGGASYADSVRGRFTISRENAKNAVYLEMNSLKPEDTAVYYCAARAPTTQEYDYWGQGTQVTVSSEPKSSDKTHTCPPCPAPELLGGPSVFLFPPKPKDTLMISRTPEVTCVVVDVSHEDPEVKFNWYVDGVEVHNAKTKPREEQYNSTYRVVSVLTVLHQDWLNGKEYKCKVSNKALPAPIEKTISKAKGQPREPQVYTLPPSRDELTKNQVSLTCLVKGFYPSDIAVEWESNGQPENNYKTTPPVLDSDGSFFLYSKLTVDKSRWQQGNVFSCSVMHEALHNHYTQKSLSLSPGK

SEQ ID NO: 136 - protein, 355 aa, VHH27-Fc
QLQLVESGGDLVQPGESLRLSCVASGRTLSTYEIGWFRQAPGKEREGVSCVTPTGFGTSYADSVRGRFTISRENAKNAVYLEMNSLKPEDTAVYYCAGSGKGLGSLQRSPDDWGQGTQVTVSSEPKSSDKTHTCPPCPAPELLGGPSVFLFPPKPKDTLMISRTPEVTCVVVDVSHEDPEVKFNWYVDGVEVHNAKTKPREEQYNSTYRVVSVLTVLHQDWLNGKEYKCKVSNKALPAPIEKTISKAKGQPREPQVYTLPPSRDELTKNQVSLTCLVKGFYPSDIAVEWESNGQPENNYKTTPPVLDSDGSFFLYSKLTVDKSRWQQGNVFSCSVMHEALHNHYTQKSLSLSPGK

SEQ ID NO: 137 - DNA, 705 bp, Fc
cgtacggagcccaaatcttgtgacaaaactcacacatgcccaccgtgcccagcacctgaactcctggggggaccgtcagtcttcctcttccccccaaaacccaaggacaccctcatgatctcccggacccctgaggtcacatgcgtggtggtggacgtgagccacgaagaccctgaggtcaagttcaactggtacgtggacggcgtggaggtgcataatgccaagacaaagccgcgggaggagcagtacaacagcacgtaccgtgtggtcagcgtcctcaccgtcctgcaccaggactggctgaatggcaaggagtacaagtgcaaggtctccaacaaagccctcccagcccccatcgagaaaaccatctccaaagccaaagggcagccccgagaaccacaggtgtacaccctgcccccatcccgggatgagctgaccaagaaccaggtcagcctgacctgcctggtcaaaggcttctatcccagcgacatcgccgtggagtgggagagcaatgggcagccggagaacaactacaagaccacgcctcccgtgctggactccgacggctccttcttcctctacagcaagctcaccgtggacaagagcaggtggcagcaggggaacgtcttctcatgctccgtgatgcatgaggctctgcacaaccactacacgcagaagagcctctccctgtctccgggtaaatga

SEQ ID NO: 138 - DNA, 23 bp, Primer For-1
gtcctggctgctcttctacaagg

SEQ ID NO: 139 - DNA, 23 bp, Primer Rev-1
ggtacgtgctgttgaactgttcc

SEQ ID NO: 140 - DNA, 32 bp, Primer For-2
ctagtgcggccgctggagacggtgacctgggt

SEQ ID NO: 141 - DNA, 29 bp, Primer Rev-2
gatgtgcagctgcaggagtctggrggagg

SEQ ID NO: 142 - DNA, 21 bp, RBD-qF1
caatggtttaacaggcacagg

SEQ ID NO: 143 - DNA, 21 bp, RBD-qR1
ctcaagtgtctgtggatcacg